European Patent Specification EP 3 591 041 B1, published April 30, 2025. Title: Anti-tumor composition comprising oncolytic adenovirus and immune checkpoint inhibitor. Applicant: Industry-university Cooperation Foundation Hanyang University. The sequence listing filed with the application follows.

SEQUENCE LISTING (9 sequences)

SEQ ID NO: 1 - DNA, 648 bp, IL-12A
atgtgtcaatcacgctacctcctctttttggccacccttgccctcctaaaccacctcagtttggccagggtcattccagtctctggacctgccaggtgtcttagccagtcccgaaacctgctgaagaccacagatgacatggtgaagacggccagagaaaaactgaaacattattcctgcactgctgaagacatcgatcatgaagacatcacacgggaccaaaccagcacattgaagacctgtttaccactggaactacacaagaacgagagttgcctggctactagagagacttcttccacaacaagagggagctgcctgcccccacagaagacgtctttgatgatgaccctgtgccttggtagcatctatgaggacttgaagatgtaccagacagagttccaggccatcaacgcagcacttcagaatcacaaccatcagcagatcattctagacaagggcatgctggtggccatcgatgagctgatgcagtctctgaatcataatggcgagactctgcgccagaaacctcctgtgggagaagcagacccttacagagtgaaaatgaagctctgcatcctgcttcacgccttcagcacccgcgtcgtgaccatcaacagggtgatgggctatctgagctccgcctga

SEQ ID NO: 2 - DNA, 1008 bp, IL-12B
atgtgtcctcagaagctaaccatctcctggtttgccatcgttttgctggtgtctccactcatggccatgtgggagctggagaaagacgtttatgttgtagaggtggactggactcccgatgcccctggagaaacagtgaacctcacctgtgacacgcctgaagaagatgacatcacctggacctcagaccagagacatggagtcataggctctggaaagaccctgaccatcactgtcaaagagtttctagatgctggccagtacacctgccacaaaggaggcgagactctgagccactcacatctgctgctccacaagaaggaaaatggaatttggtccactgaaattttaaaaaatttcaaaaacaagactttcctgaagtgtgaagcaccaaattactccggacggttcacgtgctcatggctggtgcaaagaaacatggacttgaagttcaacatcaagagcagtagcagttcccctgactctcgggcagtgacatgtggaatggcgtctctgtctgcagagaaggtcacactggaccaaagggactatgagaagtattcagtgtcctgccaggaggatgtcacctgcccaactgccgaggagaccctgcccattgaactggcgttggaagcacggcagcagaataaatatgagaactacagcaccagcttcttcatcagggacatcatcaaaccagacccgcccaagaacttgcagatgaagcctttgaagaactcacaggtggaggtcagctgggagtaccctgactcctggagcactccccattcctacttctccctcaagttctttgttcgaatccagcgcaagaaagaaaagatgaaggagacagaggaggggtgtaaccagaaaggtgcgttcctcgtagagaagacatctaccgaagtccaatgcaaaggcgggaatgtctgcgtgcaagctcaggatcgctattacaattcctcatgcagcaagtgggcatgtgttccctgcagggtccgatcctag

SEQ ID NO: 3 - DNA, 597 bp, IRES
tagcgatccgcccctctccctcccccccccctaacgttactggccgaagccgcttggaataaggccggtgtgcgtttgtctatatgttattttccaccatattgccgtcttttggcaatgtgagggcccggaaacctggccctgtcttcttgacgagcattcctaggggtctttcccctctcgccaaaggaatgcaaggtctgttgaatgtcgtgaaggaagcagttcctctggaagcttcttgaagacaaacaacgtctgtagcgaccctttgcaggcagcggaaccccccacctggcgacaggtgcctctgcggccaaaagccacgtgtataagatacacctgcaaaggcggcacaaccccagtgccacgttgtgagttggatagttgtggaaagagtcaaatggctctcctcaagcgtattcaacaaggggctgaaggatgcccagaaggtaccccattgtatgggatctgatctggggcctcggtacacatgctttacatgtgtttagtcgaggttaaaaaaacgtctaggcccccgaaccacggggacgtggttttccttttgaaaaacacgatgataatatggccacaacc

SEQ ID NO: 4 - DNA, 426 bp, GM-CSF
atgtggctgcagaatttacttttcctgggcattgtggtctacagcctctcagcacccacccgctcacccatcactgtcacccggccttggaagcatgtagaggccatcaaagaagccctgaacctcctggatgacatgcctgtcacattgaatgaagaggtagaagtcgtctctaacgagttctccttcaagaagctaacatgtgtgcagacccgcctgaagatattcgagcagggtctacggggcaatttcaccaaactcaagggcgccttgaacatgacagccagctactaccagacatactgccccccaactccggaaacggactgtgaaacacaagttaccacctatgcggatttcatagacagccttaaaacctttctgactgatatcccctttgaatgcaaaaaaccagtccaaaaatga

SEQ ID NO: 5 - DNA, 558 bp, Relaxin
atgcctcgcctgttcttgttccacctgctagaattctgtttactactgaaccaattttccagagcagtcgcggccaaatggaaggacgatgttattaaattatgcggccgcgaattagttcgcgcgcagattgccatttgcggcatgagcacctggagcaaaaggtctctgagccaggaagatgctcctcagacacctagaccagtggcagaaattgtaccatccttcatcaacaaagatacagaaactataattatcatgttggaattcattgctaatttgccaccggagctgaaggcagccctatctgagaggcaaccatcattaccagagctacagcagtatgtacctgcattaaaggattccaatcttagctttgaagaatttaagaaacttattcgcaataggcaaagtgaagccgcagacagcaatccttcagaattaaaatacttaggcttggatactcattctcaaaaaaagagacgaccctacgtggcactgtttgagaaatgttgcctaattggttgtaccaaaaggtctcttgctaaatattgctga

SEQ ID NO: 6 - DNA, 441 bp, Murine VEGF mRNA sequence
atgaactttctgctctcttgggtgcactggaccctggctttactgctgtacctccaccatgccaagtggtcccaggctgcacccacgacagaaggagagcagaagtcccatgaagtgatcaagttcatggatgtctaccagcgaagctactgccgtccgattgagaccctggtggacatcttccaggagtaccccgacgagatagagtacatcttcaagccgtcctgtgtgccgctgatgcgctgtgcaggctgctgtaacgatgaagccctggagtgcgtgcccacgtcagagagcaacatcaccatgcagatcatgcggatcaaacctcaccaaagccagcacataggagagatgagcttcctacagcacagcagatgtgaatgcagaccaaagaaagacagaacaaagccagaaaaatgtgacaagccaaggcggtga

SEQ ID NO: 7 - DNA, 576 bp, Homo sapiens VEGF mRNA
atgaactttctgctgtcttgggtgcattggagccttgccttgctgctctacctccaccatgccaagtggtcccaggctgcacccatggcagaaggaggggggcagaatcatcacgaagtggtgaagttcatggatgtctatcagcgcagctactgccatccaatcgagaccctggtggacatcttccaggagtaccctgatgagatcgagtacatcttcaagccatcctgtgtgcccctgatgcgatgcgggggctgctgcaatgacgagggcctggagtgtgtgcccactgaggagtccaacatcaccatgcagattatgcggatcaaacctcaccaaggccagcacataggagagatgagcttcctacagcacaacaaatgtgaatgcagaccaaagaaagatagagcaagacaagaaaatccctgtgggccttgctcagagcggagaaagcatttgtttgtacaagatccgcagacgtgtaaatgttcctgcaaaaacacagactcgcgttgcaaggcgaggcagcttgagttaaacgaacgtacttgcagatgtgacaagccgaggcggtga

SEQ ID NO: 8 - DNA, 71 bp, Artificial Sequence
  shVEGF sense
gatcccggaaggagagcagaagtcccatgttcaagagacatgggacttctgctctcctttttttttggaaa

SEQ ID NO: 9 - DNA, 71 bp, Artificial Sequence
  shVEGF anti-sense
tttccaaaaaaaaaggagagcagaagtcccatgtctcttgaacatgggacttctgctctccttccgggatc